European Patent Application EP 4 585 602 A1, published July 16, 2025. Title: COMPOUND, CONJUGATE, COMPOSITION, AND USES THEREOF. Applicant: RIGERNA THERAPEUTICS (BEIJING) CO., LTD. The sequence listing filed with the application follows.

SEQUENCE LISTING (10 sequences)

SEQ ID NO: 1 - RNA, 19 nt, synthetic construct
  source 1..19: mol_type = other RNA
  modified_base 1: mod_base = OTHER; note = 2'-methoxy and 5'-phosphorothioate bond
  modified_base 2: mod_base = OTHER; note = 2'-methoxy and 5'-phosphorothioate bond
  modified_base 3: mod_base = OTHER; note = 2'-methoxy
  modified_base 4: mod_base = OTHER; note = 2'-methoxy
  modified_base 5: mod_base = OTHER; note = 2'-methoxy
  modified_base 6: mod_base = OTHER; note = 2'-methoxy
  modified_base 7: mod_base = OTHER; note = 2 '-fluoro
  modified_base 8: mod_base = OTHER; note = 2 '-fluoro
  modified_base 9: mod_base = OTHER; note = 2 '-fluoro
  modified_base 10: mod_base = OTHER; note = 2'-methoxy
  modified_base 11: mod_base = OTHER; note = 2'-methoxy
  modified_base 12: mod_base = OTHER; note = 2'-methoxy
  modified_base 13: mod_base = OTHER; note = 2'-methoxy
  modified_base 14: mod_base = OTHER; note = 2'-methoxy
  modified_base 15: mod_base = OTHER; note = 2'-methoxy
  modified_base 16: mod_base = OTHER; note = 2'-methoxy
  modified_base 17: mod_base = OTHER; note = 2'-methoxy
  modified_base 18: mod_base = OTHER; note = 2'-methoxy
  modified_base 19: mod_base = OTHER; note = 2'-methoxy
ttttaatcctcactctaaa

SEQ ID NO: 2 - RNA, 21 nt, synthetic construct
  source 1..21: mol_type = other RNA
  modified_base 1: mod_base = OTHER; note = 2'-methoxy and 5'-phosphorothioate bond
  modified_base 2: mod_base = OTHER; note = 2 '-fluoro and 5'-phosphorothioate bond
  modified_base 3: mod_base = OTHER; note = 2'-methoxy
  modified_base 4: mod_base = OTHER; note = 2'-methoxy
  modified_base 5: mod_base = OTHER; note = 2'-methoxy
  modified_base 6: mod_base = OTHER; note = 2 '-fluoro
  modified_base 7: mod_base = OTHER; note = 2'-methoxy
  modified_base 8: mod_base = OTHER; note = 2'-methoxy
  modified_base 9: mod_base = OTHER; note = 2'-methoxy
  modified_base 10: mod_base = OTHER; note = 2'-methoxy
  modified_base 11: mod_base = OTHER; note = 2'-methoxy
  modified_base 12: mod_base = OTHER; note = 2'-methoxy
  modified_base 13: mod_base = OTHER; note = 2'-methoxy
  modified_base 14: mod_base = OTHER; note = 2 '-fluoro
  modified_base 15: mod_base = OTHER; note = 2'-methoxy
  modified_base 16: mod_base = OTHER; note = 2 '-fluoro
  modified_base 17: mod_base = OTHER; note = 2'-methoxy
  modified_base 18: mod_base = OTHER; note = 2'-methoxy
  modified_base 19: mod_base = OTHER; note = 2'-methoxy and 5'-phosphorothioate bond
  modified_base 20: mod_base = OTHER; note = 2'-methoxy and 5'-phosphorothioate bond
  modified_base 21: mod_base = OTHER; note = 2'-methoxy
tttagagtgaggattaaaatg

SEQ ID NO: 3 - RNA, 19 nt, synthetic construct
  source 1..19: mol_type = other RNA
  modified_base 1: mod_base = OTHER; note = 2'-methoxy and 5'-phosphorothioate bond
  modified_base 2: mod_base = OTHER; note = 2'-methoxy and 5'-phosphorothioate bond
  modified_base 3: mod_base = OTHER; note = 2'-methoxy
  modified_base 4: mod_base = OTHER; note = 2'-methoxy
  modified_base 5: mod_base = OTHER; note = 2'-methoxy
  modified_base 6: mod_base = OTHER; note = 2'-methoxy
  modified_base 7: mod_base = OTHER; note = 2 '-fluoro
  modified_base 8: mod_base = OTHER; note = 2 '-fluoro
  modified_base 9: mod_base = OTHER; note = 2 '-fluoro
  modified_base 10: mod_base = OTHER; note = 2'-methoxy
  modified_base 11: mod_base = OTHER; note = 2'-methoxy
  modified_base 12: mod_base = OTHER; note = 2'-methoxy
  modified_base 13: mod_base = OTHER; note = 2'-methoxy
  modified_base 14: mod_base = OTHER; note = 2'-methoxy
  modified_base 15: mod_base = OTHER; note = 2'-methoxy
  modified_base 16: mod_base = OTHER; note = 2'-methoxy
  modified_base 17: mod_base = OTHER; note = 2'-methoxy
  modified_base 18: mod_base = OTHER; note = 2'-methoxy
  modified_base 19: mod_base = OTHER; note = 2'-methoxy
ccaagagcaccaagaacta

SEQ ID NO: 4 - RNA, 21 nt, synthetic construct
  source 1..21: mol_type = other RNA
  modified_base 1: mod_base = OTHER; note = 2'-methoxy and 5'-phosphorothioate bond
  modified_base 2: mod_base = OTHER; note = 2 '-fluoro and 5'-phosphorothioate bond
  modified_base 3: mod_base = OTHER; note = 2'-methoxy
  modified_base 4: mod_base = OTHER; note = 2'-methoxy
  modified_base 5: mod_base = OTHER; note = 2'-methoxy
  modified_base 6: mod_base = OTHER; note = 2 '-fluoro
  modified_base 7: mod_base = OTHER; note = 2'-methoxy
  modified_base 8: mod_base = OTHER; note = 2'-methoxy
  modified_base 9: mod_base = OTHER; note = 2'-methoxy
  modified_base 10: mod_base = OTHER; note = 2'-methoxy
  modified_base 11: mod_base = OTHER; note = 2'-methoxy
  modified_base 12: mod_base = OTHER; note = 2'-methoxy
  modified_base 13: mod_base = OTHER; note = 2'-methoxy
  modified_base 14: mod_base = OTHER; note = 2 '-fluoro
  modified_base 15: mod_base = OTHER; note = 2'-methoxy
  modified_base 16: mod_base = OTHER; note = 2 '-fluoro
  modified_base 17: mod_base = OTHER; note = 2'-methoxy
  modified_base 18: mod_base = OTHER; note = 2'-methoxy
  modified_base 19: mod_base = OTHER; note = 2'-methoxy and 5'-phosphorothioate bond
  modified_base 20: mod_base = OTHER; note = 2'-methoxy and 5'-phosphorothioate bond
  modified_base 21: mod_base = OTHER; note = 2'-methoxy
tagttcttggtgctcttggtt

SEQ ID NO: 5 - DNA, 20 bp, synthetic construct
  source 1..20: mol_type = other DNA
gggttccacgtccatcagta

SEQ ID NO: 6 - DNA, 20 bp, synthetic construct
  source 1..20: mol_type = other DNA
acaccgtcctttccagcagt

SEQ ID NO: 7 - DNA, 19 bp, synthetic construct
  source 1..19: mol_type = other DNA
tgcaccaccaactgcttag

SEQ ID NO: 8 - DNA, 19 bp, synthetic construct
  source 1..19: mol_type = other DNA
ggatgcagggatgatgttc

SEQ ID NO: 9 - DNA, 23 bp, synthetic construct
  source 1..23: mol_type = other DNA
gaggagcagctaaccaacttaat

SEQ ID NO: 10 - DNA, 23 bp, synthetic construct
  source 1..23: mol_type = other DNA
tctgcatgtgctgttgacttaat